European Patent Specification EP 2 884 994 B1, published January 18, 2023. Title: A composition for treating hyperlipidemia comprising oxyntomodulin derivative. Applicant: HANMI PHARM. CO., LTD. The sequence listing filed with the application follows.

SEQUENCE LISTING (53 sequences)

SEQ ID NO: 1 - protein, 37 aa, Homo sapiens
  oxyntomodulin
HSQGTFTSDYSKYLDSRRAQDFVQWLMNTKRNRNNIA

SEQ ID NO: 2 - protein, 37 aa, Artificial Sequence
  oxyntomodulin derivative
  VARIANT (1): Xaa = 4-imidazoacetyl
XSQGTFTSDYSKYLDEEAVRLFIEWLMNTKRNRNNIA

SEQ ID NO: 3 - protein, 39 aa, Artificial Sequence
  oxyntomodulin derivative
  VARIANT (1): Xaa = 4-imidazoacetyl
XSQGTFTSDYSKYLDERRAQDFVAWLKNTGPSSGAPPPS

SEQ ID NO: 4 - protein, 39 aa, Artificial Sequence
  oxyntomodulin derivative
  VARIANT (1): Xaa = 4-imidazoacetyl
XGQGTFTSDYSRYLEEEAVRLFIEWLKNGGPSSGAPPPS

SEQ ID NO: 5 - protein, 39 aa, Artificial Sequence
  oxyntomodulin derivative
  VARIANT (1): Xaa = 4-imidazoacetyl
XGQGTFTSDYSRQMEEEAVRLFIEWLKNGGPSSGAPPPS

SEQ ID NO: 6 - protein, 42 aa, Artificial Sequence
  oxyntomodulin derivative
  VARIANT (1): Xaa = 4-imidazoacetyl
XGEGTFTSDLSRQMEEEAVRLFIEWAAHSQGTFTSDYSKYLD

SEQ ID NO: 7 - protein, 30 aa, Artificial Sequence
  oxyntomodulin derivative
  VARIANT (1): Xaa = 4-imidazoacetyl
XSQGTFTSDYSRYLDEEAVRLFIEWLMNTK

SEQ ID NO: 8 - protein, 29 aa, Artificial Sequence
  oxyntomodulin derivative
  VARIANT (1): Xaa = 4-imidazoacetyl
XSQGTFTSDLSRQLEEEAVRLFIEWLMNK

SEQ ID NO: 9 - protein, 37 aa, Artificial Sequence
  oxyntomodulin derivative
  VARIANT (1): Xaa = 4-imidazoacetyl
  VARIANT (20): Xaa = alpha-methyl-glutamic acid
XGQGTFTSDYSRYLDEEAVXLFIEWLMNTKRNRNNIA

SEQ ID NO: 10 - protein, 40 aa, Artificial Sequence
  oxyntomodulin derivative
  VARIANT (1): Xaa = 4-imidazoacetyl
XSQGTFTSDYSRQMEEEAVRLFIEWLMNGGPSSGAPPPSK

SEQ ID NO: 11 - protein, 43 aa, Artificial Sequence
  oxyntomodulin derivative
  VARIANT (1): Xaa = 4-imidazoacetyl
XGEGTFTSDLSRQMEEEAVRLFIEWAAHSQGTFTSDYSRYLDK

SEQ ID NO: 12 - protein, 38 aa, Artificial Sequence
  oxyntomodulin derivative
  VARIANT (1): Xaa = 4-imidazoacetyl
XSQGTFTSDYSRYLDGGGHGEGTFTSDLSKQMEEEAVK

SEQ ID NO: 13 - protein, 30 aa, Artificial Sequence
  oxyntomodulin derivative
  VARIANT (1): Xaa = 4-imidazoacetyl
  VARIANT (16): Xaa = alpha-methyl-glutamic acid
  VARIANT (20): Xaa = alpha-methyl-glutamic acid
XSQGTFTSDYSRYLDXEAVXLFIEWLMNTK

SEQ ID NO: 14 - protein, 37 aa, Artificial Sequence
  oxyntomodulin derivative
  VARIANT (1): Xaa = 4-imidazoacetyl
  VARIANT (20): Xaa = alpha-methyl-glutamic acid
  VARIANT (24): Xaa = alpha-methyl-glutamic acid
XGQGTFTSDYSRYLDEEAVXLFIXWLMNTKRNRNNIA

SEQ ID NO: 15 - protein, 37 aa, Artificial Sequence
  oxyntomodulin derivative
  VARIANT (1): Xaa = 4-imidazoacetyl
  VARIANT (24): Xaa = alpha-methyl-glutamic acid
XGQGTFTSDYSRYLDEEAVRLFIXWLMNTKRNRNNIA

SEQ ID NO: 16 - protein, 34 aa, Artificial Sequence
  oxyntomodulin derivative
  VARIANT (1): Xaa = 4-imidazoacetyl
XSQGTFTSDLSRQLEGGGHSQGTFTSDLSRQLEK

SEQ ID NO: 17 - protein, 37 aa, Artificial Sequence
  oxyntomodulin derivative
  VARIANT (1): Xaa = 4-imidazoacetyl
XSQGTFTSDYSRYLDEEAVRLFIEWIRNTKRNRNNIA

SEQ ID NO: 18 - protein, 40 aa, Artificial Sequence
  oxyntomodulin derivative
  VARIANT (1): Xaa = 4-imidazoacetyl
XSQGTFTSDYSRYLDEEAVRLFIEWIRNGGPSSGAPPPSK

SEQ ID NO: 19 - protein, 37 aa, Artificial Sequence
  oxyntomodulin derivative
  VARIANT (1): Xaa = 4-imidazoacetyl
  VARIANT (16), (20): amino acids at position 16 and position 20 form a ring
XSQGTFTSDYSRYLDEEAVKLFIEWIRNTKRNRNNIA

SEQ ID NO: 20 - protein, 40 aa, Artificial Sequence
  oxyntomodulin derivative
  VARIANT (1): Xaa = 4-imidazoacetyl
  VARIANT (16), (20): amino acids at position 16 and position 20 form a ring
XSQGTFTSDYSRYLDEEAVKLFIEWIRNGGPSSGAPPPSK

SEQ ID NO: 21 - protein, 37 aa, Artificial Sequence
  oxyntomodulin derivative
  VARIANT (1): Xaa = 4-imidazoacetyl
XSQGTFTSDYSRQLEEEAVRLFIEWVRNTKRNRNNIA

SEQ ID NO: 22 - protein, 30 aa, Artificial Sequence
  oxyntomodulin derivative
  VARIANT (1): Xaa = desamino-histidyl.
  VARIANT (16), (20): amino acids at position 16 and position 20 form a ring
XSQGTFTSDYSKYLDEKRAKEFVQWLMNTK

SEQ ID NO: 23 - protein, 29 aa, Artificial Sequence
  oxyntomodulin derivative
  VARIANT (2): Xaa = aminoisobutyric acid
HXQGTFTSDYSKYLDEKRAKEFVCWLMNT

SEQ ID NO: 24 - protein, 30 aa, Artificial Sequence
  oxyntomodulin derivative
  VARIANT (2): Xaa = aminoisobutyric acid
HXQGTFTSDYSKYLDEKRAKEFVQWLMNTC

SEQ ID NO: 25 - protein, 30 aa, Artificial Sequence; identical to SEQ ID NO: 24
  oxyntomodulin derivative
  VARIANT (2): Xaa = aminoisobutyric acid
  VARIANT (16), (20): amino acids at position 16 and position 20 form a ring

SEQ ID NO: 26 - protein, 30 aa, Artificial Sequence; identical to SEQ ID NO: 24
  oxyntomodulin derivative
  VARIANT (2): Xaa = aminoisobutyric acid
  VARIANT (12), (16): amino acids at position 12 and position 16 form a ring

SEQ ID NO: 27 - protein, 29 aa, Artificial Sequence
  oxyntomodulin derivative
  VARIANT (2): Xaa = aminoisobutyric acid
  VARIANT (16), (20): amino acids at position 16 and position 20 form a ring
HXQGTFTSDYSKYLDEQAAKEFICWLMNT

SEQ ID NO: 28 - protein, 29 aa, Artificial Sequence
  oxyntomodulin derivative
  VARIANT (2): Xaa = aminoisobutyric acid
HXQGTFTSDYSKYLDEKRAKEFVQWLMNT

SEQ ID NO: 29 - protein, 37 aa, Artificial Sequence
  oxyntomodulin derivative
  VARIANT (2): Xaa = d-serine.
HXQGTFTSDYSKYLDSRRAQDFVQWLMNTKRNRNNIA

SEQ ID NO: 30 - protein, 37 aa, Artificial Sequence
  oxyntomodulin derivative
  VARIANT (1): Xaa = 4-imidazoacetyl
XSQGTFTSDYSKYLDSRRAQDFVQWLMNTKRNRNNIA

SEQ ID NO: 31 - protein, 37 aa, Artificial Sequence
  oxyntomodulin derivative
  VARIANT (1): Xaa = 4-imidazoacetyl
  VARIANT (2): Xaa = d-serine.
XXQGTFTSDYSKYLDSRRAQDFVQWLMNTKRNRNNIA

SEQ ID NO: 32 - protein, 30 aa, Artificial Sequence
  oxyntomodulin derivative
  VARIANT (1): Xaa = 4-imidazoacetyl
  VARIANT (2): Xaa = aminoisobutyric acid
XXQGTFTSDYSKYLDEKRAKEFVQWLMNTC

SEQ ID NO: 33 - protein, 30 aa, Artificial Sequence
  oxyntomodulin derivative
  VARIANT (2): Xaa = aminoisobutyric acid
HXQGTFTSDYAKYLDEKRAKEFVQWLMNTC

SEQ ID NO: 34 - protein, 30 aa, Artificial Sequence
  oxyntomodulin derivative
  VARIANT (2): Xaa = aminoisobutyric acid
YXQGTFTSDYSKYLDEKRAKEFVQWLMNTC

SEQ ID NO: 35 - protein, 8 aa, Artificial Sequence
  group R2
KRNRNNIA

SEQ ID NO: 36 - protein, 10 aa, Artificial Sequence
  group R2
GPSSGAPPPS

SEQ ID NO: 37 - protein, 11 aa, Artificial Sequence
  group R2
GPSSGAPPPSK

SEQ ID NO: 38 - protein, 15 aa, Artificial Sequence
  group R2
HSQGTFTSDYSKYLD

SEQ ID NO: 39 - protein, 16 aa, Artificial Sequence
  group R2
HSQGTFTSDYSRYLDK

SEQ ID NO: 40 - protein, 20 aa, Artificial Sequence
  group R2
HGEGTFTSDLSKQMEEEAVK

SEQ ID NO: 41 - protein, 28 aa, Artificial Sequence
  group A or B
SQGTFTSDYSKYLDSRRAQDFVQWLMNT

SEQ ID NO: 42 - protein, 28 aa, Artificial Sequence
  group A or B
SQGTFTSDYSKYLDEEAVRLFIEWLMNT

SEQ ID NO: 43 - protein, 28 aa, Artificial Sequence
  group A or B
SQGTFTSDYSKYLDERRAQDFVAWLKNT

SEQ ID NO: 44 - protein, 28 aa, Artificial Sequence
  group A or B
GQGTFTSDYSRYLEEEAVRLFIEWLKNG

SEQ ID NO: 45 - protein, 28 aa, Artificial Sequence
  group A or B
GQGTFTSDYSRQMEEEAVRLFIEWLKNG

SEQ ID NO: 46 - protein, 26 aa, Artificial Sequence
  group A or B
GEGTFTSDLSRQMEEEAVRLFIEWAA

SEQ ID NO: 47 - protein, 28 aa, Artificial Sequence
  group A or B
SQGTFTSDYSRQMEEEAVRLFIEWLMNG

SEQ ID NO: 48 - protein, 24 aa, Artificial Sequence
  group B
GEGTFTSDLSRQMEEEAVRLFIEW

SEQ ID NO: 49 - protein, 14 aa, Artificial Sequence
  group B
SQGTFTSDYSRYLD

SEQ ID NO: 50 - DNA, 30 bp, Artificial Sequence
  primer
cccggcccccgcggccgctattcgaaatac

SEQ ID NO: 51 - DNA, 33 bp, Artificial Sequence
  primer
gaacggtccggaggacgtcgactcttaagatag

SEQ ID NO: 52 - DNA, 34 bp, Artificial Sequence
  primer
cagcgacaccgaccgtccccccgtacttaaggcc

SEQ ID NO: 53 - DNA, 32 bp, Artificial Sequence
  primer
ctaaccgactctcggggaagactgagctcgcc